European Patent Specification EP 3 679 132 B1, published February 21, 2024. Title: Leistungsverbesserte Proteasen III. Applicant: Henkel AG & Co. KGaA. The sequence listing filed with the application follows.

SEQUENCE LISTING (5 sequences)

SEQ ID NO: 1 - protein, 275 aa, Bacillus pumilus
AQTVPYGIPQIKAPAVHAQGYKGANVKVAVLDTGIHAAHPDLNVAGGASFVPSEPNATQDFQSHGTHVAGTIAALDNTIGVLGVAPSASLYAVKVLDRNGDGQYSWIISGIEWAVANNMDVINMSLGGPNGSTALKNAVDTANNRGVVVVAAAGNSGSTGSTSTVGYPAKYDSTIAVANVNSSNVRNSSSSAGPELDVSAPGTSILSTVPSSGYTSYTGTSMASPHVAGAAALILSKNPNLSNSQVRQRLENTATPLGNSFYYGKGLINAQAASN

SEQ ID NO: 2 - protein, 275 aa, Artificial Sequence
  Mutationsvariante von B. pumilus Protease
AQTVPYGIPQIKAPAVHAQGYKGANVKVAVLDTGIHAAHPDLNVAGGASFVPSEPNATQDFQSHGTHVAGTIAALDNTIGVLGVAPSASLYAVKVLDRNGEGQYSWIISGIEWAVANNMDVINMSLGGPDGSRALKNAVDTANNRGVVVVAAAGNSGSTGSTSTVGYPAKYDSTIAVANVNSSNVRNSSSSAGPELDVSAPGTSILSTVPSSGYTSYTGTSMAAPHVAGAAALILSKNPNLSNSQVRQRLENTATPLGNSFYYGKGLINAEAASN

SEQ ID NO: 3 - protein, 275 aa, Artificial Sequence
  Mutationsvariante von B. pumilus Protease
AQTVPYGIPQIKAPAVHAQGYKGANVKVAVLDTGIHAAHPDLNVAGGASFVPSEPNATQDFQSHGTHVAGTIAALDNTIGVLGVAPSASLYAVKVLDRNGEGQYSWIISGIEWAVANNMDVINMSLGGPDGSTALKNAVDTANKRGVVVVAAAGNSGSTGSTSTVGYPAKYDSTIAVANVNSSNVRNSSSSAGPELDVSAPGTSILSTVPSSGYTSYTGTSMASPHVAGAAALILSKNPNLSNSQVRQRLETTATPLGNSFYYGKGLINAEAASN

SEQ ID NO: 4 - protein, 275 aa, Artificial Sequence
  Mutationsvariante von B. pumilus Protease
AQTVPYGIPQIKAPAVHAQGYKGANVKVAVLDTGIHAAHPDLNVAGGASFVPSEPNATQDFQSHGTHVAGTIAALDNTIGVLGVAPSASLYAVKVLDRNGDGQYSWIISGIEWAVANNMDVINMSLGGPDGSTALKNAVDTANKRGVVVVAAAGNSGSTGSTSTVGYPAKYDSTIAVANVNSSNVRNSSSSAGPELDVSAPGTSILSTVPSSGYTSYTGTSMASPHVAGAAALILSKNPNLSNSQVRQRLETTATPLGNSFYYGKGLINAEAASN

SEQ ID NO: 5 - protein, 275 aa, Artificial Sequence
  Mutationsvariante von B. pumilus Protease
AQTVPYGIPQIKAPAVHAQGYKGANVKVAVLDTGIHAAHPDLNVAGGASFVPSEPNATQDFQSHGTHVAGTIAALDNTIGVLGVAPSASLYAVKVLDRNGDGQYSWIISGIEWAVANNMDVINMSLGGPDGSRALKNAVDTANNRGVVVVAAAGNSGSTGSTSTVGYPAKYDSTIAVANVNSSNVRNSSSSAGPELDVSAPGTSILSTVPSSGYTSYTGTSMAAPHVAGAAALILSKNPNLSNSQVRQRLENTATPLGNSFYYGKGLINAEAASN